European Patent Specification EP 2 632 434 B1, published August 20, 2025. Title: Preparation of an antigenic construct. Applicant: AC Immune S.A. et al. The sequence listing filed with the application follows.

SEQUENCE LISTING (12 sequences)

SEQ ID NO: 1 - protein, 30 aa, Homo sapiens
  VARIANT (18)..(18): /replace="phosphorylated Serine"
  VARIANT (26)..(26): /replace="phosphorylated Serine"
RENAKAKTDHGAEIVYKSPVVSGDTSPRHL

SEQ ID NO: 2 - protein, 16 aa, Homo sapiens
  VARIANT (14)..(14): /replace="phosphorylated Tyrosin"
RQEFEVMEDHAGTYGL

SEQ ID NO: 3 - protein, 16 aa, Homo sapiens
  VARIANT (7)..(7): /replace="phosphorylated Threonine"
  VARIANT (9)..(9): /replace="phosphorylated Serine"
PGSRSRTPSLPTPPTR

SEQ ID NO: 4 - protein, 16 aa, Homo sapiens
  VARIANT (7)..(7): /replace="phosphorylated Serine"
  VARIANT (10)..(10): /replace="phosphorylated Threonine"
GYSSPGSPGTPGSRSR

SEQ ID NO: 5 - protein, 16 aa, Homo sapiens
  VARIANT (4)..(4): /replace="phosphorylated Serine"
  VARIANT (12)..(12): /replace="phosphorylated Serine"
VYKSPVVSGDTSPRHL

SEQ ID NO: 6 - protein, 18 aa, Homo sapiens
  VARIANT (4)..(4): /replace="phosphorylated Serine"
  VARIANT (9)..(9): /replace="phosphorylated Serine"
GDTSPRHLSNVSSTGSID

SEQ ID NO: 7 - protein, 17 aa, Homo sapiens
  VARIANT (3)..(3): /replace="phosphorylated Serine"
  VARIANT (6)..(6): /replace="phosphorylated Threonine"
  VARIANT (13)..(13): /replace="phosphorylated Threonine"
  VARIANT (15)..(15): /replace="phosphorylated Serine"
PGSPGTPGSRSRTPSLP

SEQ ID NO: 8 - protein, 12 aa, Homo sapiens
  VARIANT (3)..(3): /replace="phosphorylated Serine"
HLSNVSSTGSID

SEQ ID NO: 9 - protein, 10 aa, Homo sapiens
  VARIANT (6)..(6): /replace="phosphorylated Serine"
VSGDTSPRHL

SEQ ID NO: 10 - protein, 15 aa, Homo sapiens
DAEFRHDSGYEVHHQ

SEQ ID NO: 11 - protein, 19 aa, Homo sapiens
  VARIANT (1)..(1): /replace="acetylated Lysine"
  VARIANT (2)..(2): /replace="acetylated Lysine"
  VARIANT (18)..(18): /replace="acetylated Lysine"
  VARIANT (19)..(19): /replace="acetylated Lysine"
KKDAEFRHDSGYEVHHQKK

SEQ ID NO: 12 - protein, 19 aa, Homo sapiens
  VARIANT (1)..(1): /replace="palmitoylated Lysine"
  VARIANT (2)..(2): /replace="palmitoylated Lysine"
  VARIANT (18)..(18): /replace="palmitoylated Lysine"
  VARIANT (19)..(19): /replace="palmitoylated Lysine"
KKDAEFRHDSGYEVHHQKK